European Patent Specification EP 3 180 361 B1, published January 8, 2025. Title: RECOMBINANT ANTIBODY MOLECULES FOR TARGET CELL RESTRICTED T CELL ACTIVATION. Applicant: Eberhard Karls Universitaet Tuebingen Universitaet Wuerzburg Deutsches Krebsforschungszentrum. The sequence listing filed with the application follows.

SEQUENCE LISTING (127 sequences)

SEQ ID NO: 1 - protein, 107 aa, Artificial Sequence
  anti-FLT3 chimeric single variable domain  light chain (clone 4G8) (VL)
DIVLTQSPATLSVTPGDSVSLSCRASQSISNNLHWYQQKSHESPRLLIKYASQSISGIPSRFSGSGSGTDFTLSINSVETEDFGVYFCQQSNTWPYTFGGGTKLEIK

SEQ ID NO: 2 - protein, 118 aa, Artificial Sequence
  anti-FLT3 chimeric single variable domain heavy chain (clone 4G8) (VH)
QVQLQQPGAELVKPGASLKLSCKSSGYTFTSYWMHWVRQRPGHGLEWIGEIDPSDSYKDYNQKFKDKATLTVDRSSNTAYMHLSSLTSDDSAVYYCARAITTTPFDFWGQGTTLTVSS

SEQ ID NO: 3 - protein, 107 aa, Artificial Sequence [sequence omitted]

SEQ ID NO: 4 - protein, 122 aa, Artificial Sequence [sequence omitted]

SEQ ID NO: 5 - protein, 113 aa, Artificial Sequence
  anti-FLT3 single variable domain (clone BV10), VL
DIVMTQSPSSLSVSAGEKVTMSCKSSQSLLNSGNQKNYMAWYQQKPGQPPKLLIYGASTRESGVPDRFTGSGSGTDFTLTISSVQAEDLAVYYCQNDHSYPLTFGAGTKLELK

SEQ ID NO: 6 - protein, 123 aa, Artificial Sequence
  anti-FLT3 single variable domain VH (clone BV10)
QVQLKQSGPGLVQPSQSLSITCTVSGFSLTNYGLHWVRQSPGKGLEWLGVIWSGGSTDYNAAFISRLSISKDNSKSQVFFKMNSLQADDTAIYYCARKGGIYYANHYYAMDYWGQGTSVTVSS

SEQ ID NO: 7 - protein, 106 aa, Artificial Sequence
  C-terminal TCR /  single variable domain (clone BMA031) VL
QIVLTQSPAIMSASPGEKVTMTCSATSSVSYMHWYQQKSGTSPKRWIYDTSKLASGVPARFSGSGSGTSYSLTISSMEAEDAATYYCQQWSSNPLTFGAGTKLELK

SEQ ID NO: 8 - protein, 119 aa, Artificial Sequence
  C-terminal TCR /  single variable domain (clone BMA031 VH
EVQLQQSGPELVKPGASVKMSCKASGYKFTSYVMHWVKQKPGQGLEWIGYINPYNDVTKYNEKFKGKATLTSDKSSSTAYMELSSLTSEDSAVHYCARGSYYDYDGFVYGQGTLVTVSS

SEQ ID NO: 9 - protein, 112 aa, Artificial Sequence
  Anti-CD19 single variable domain VL (clone 4G7)
DIVMTQAAPSIPVTPGESVSISCRSSKSLLNSNGNTYLYWFLQRPGQSPQLLIYRMSNLASGVPDRFSGSGSGTAFTLRISRVEAEDVGVYYCMQHLEYPFTFGAGTKLELK

SEQ ID NO: 10 - protein, 121 aa, Artificial Sequence
  Anti-CD19 single variable domain VH (clone 4G7)
EVQLQQSGPELIKPGASVKMSCKASGYTFTSYVMHWVKQKPGQGLEWIGYINPYNDGTKYNEKFKGKATLTSDKSSSTAYMELSSLTSEDSAVYYCARGTYYYGSRVFDYWGQGTTLTVSS

SEQ ID NO: 11 - protein, 112 aa, Artificial Sequence
  Anti- CD28 single variable domain (clone 9.3) VL
DIELTQSPASLAVSLGQRATISCRASESVEYYVTSLMQWYQQKPGQPPKLLIFAASNVESGVPARFSGSGSGTNFSLNIHPVDEDDVAMYFCQQSRKVPYTFGGGTKLEIKR

SEQ ID NO: 12 - protein, 120 aa, Artificial Sequence
  Anti- CD28 single variable domain (clone 9.3) VH
QVKLQQSGPGLVTPSQSLSITCTVSGFSLSDYGVHWVRQSPGQGLEWLGVIWAGGGTNYNSALMSRKSISKDNSKSQVFLKMNSLQADDTAVYYCARDKGYSYYYSMDYWGQGTTVTVSS

SEQ ID NO: 13 - protein, 111 aa, Artificial Sequence
  Anti-CD16 single variable domain (clone 3G8) VL
DIVLTQSPASLAVSLGQRATISCKASQSVDFDGDSFMNWYQQKPGQPPKLLIYTTSNLESGIPARFSASGSGTDFTLNIHPVEEEDTATYYCQQSNEDPYTFGGGTKLEIK

SEQ ID NO: 14 - protein, 118 aa, Artificial Sequence
  Anti-CD16 single variable domain (clone 3G8) VH
QVTLKESGPGILQPSQTLSLTCSFSGFSLRTSGMGVGWIRQPSGKGLEWLAHIWWDDDKRYNPALKSRLTISKDTSSNQVFLKIASVDTADTATYYCAQINPAWFAYWGQGTLVTVSS

SEQ ID NO: 15 - protein, 111 aa, Artificial Sequence
  Anti-CSPG4 chimeric single variable domain  VL (clone 9.2.27)
DIELTQSPASLAVSLGQRATISCRASESVDSYGNSFMHWYQQKPGQPPKLLIYLASNLESGVPARFSGSGSRTDFTLTIDPVEADDAATYYCQQNNEDPLTFGGGTKLEIK

SEQ ID NO: 16 - protein, 121 aa, Artificial Sequence
  anti-CSPG4 single variable domain  VH (clone 9.2.27)
QVKLQQSGPELVKPGASVKISCKASGYAFSRSWMNWVKQRPGQGLEWIGRIYPGDGDTNYNGKFKGKATLTADKSSSTAYMQVSSLTSVDSAVYFCARGNTVVVPYTMDYWGQGTTVTVSS

SEQ ID NO: 17 - protein, 107 aa, Artificial Sequence
  Anti-EGFR single variable domain  VL(clone C225)
DILLTQSPVILSVSPGERVSFSCRASQSIGTNIHWYQQRTNGSPRLLIKYASESISGIPSRFSGSGSGTDFTLSINSVESEDIADYYCQQNNNWPTTFGAGTKLELK

SEQ ID NO: 18 - protein, 121 aa, Artificial Sequence; identical to SEQ ID NO: 16
  anti-CSPG4 single variable domain  VH (clone 9.2.27)

SEQ ID NO: 19 - protein, 98 aa, Artificial Sequence
  CH1 domain
ASTKGPSVFPLAPSSKSTSGGTAALGCLVKDYFPEPVTVSWNSGALTSGVHTFPAVLQSSGLYSLSSVVTVPSSSLGTQTYICNVNHKPSNTKVDKKV

SEQ ID NO: 20 - protein, 124 aa, Artificial Sequence
  Hinge and CH2  region
EPKSCDKTHTSPPSPAPPVAGPSVFLFPPKPKDTLMISRTPEVTCVVVGVSHEDPEVKFNWYVDGVEVHNAKTKPREEQYQSTYRVVSVLTVLHQDWLNGKEYKCKVSNKQLPSPIEKTISKAK

SEQ ID NO: 21 - protein, 107 aa, Artificial Sequence [sequence omitted]

SEQ ID NO: 22 - protein, 452 aa, Artificial Sequence
  FLT3 x CD3;  Fabv
QVQLQQPGAELVKPGASLKLSCKSSGYTFTSYWMHWVRQRPGHGLEWIGEIDPSDSYKDYNQKFKDKATLTVDRSSNTAYMHLSSLTSDDSAVYYCARAITTTPFDFWGQGTTLTVSSASTKGPSVFPLAPSSKSTSGGTAALGCLVKDYFPEPVTVSWNSGALTSGVHTFPAVLQSSGLYSLSSVVTVPSSSLGTQTYICNVNHKPSNTKVDKKVEPKSCDKTHTSPPSPAPPVAGPSVFLFPPKPKDTLMISRTPEVTCVVVGVSHEDPEVKFNWYVDGVEVHNAKTKPREEQYQSTYRVVSVLTVLHQDWLNGKEYKCKVSNKQLPSPIEKTISKAKGQPSGDIQMTQSPSSLSASVGDRVTITCRASQDIRNYLNWYQQKPGKAPKLLIYYTSRLESGVPSRFSGSGSGTDYTLTISSLQPEDFATYYCQQGNTLPWTFGQGTKVEIK

SEQ ID NO: 23 - protein, 467 aa, Artificial Sequence
  FLT3 x CD3;  Fabv
QVQLQQPGAELVKPGASLKLSCKSSGYTFTSYWMHWVRQRPGHGLEWIGEIDPSDSYKDYNQKFKDKATLTVDRSSNTAYMHLSSLTSDDSAVYYCARAITTTPFDFWGQGTTLTVSSASTKGPSVFPLAPSSKSTSGGTAALGCLVKDYFPEPVTVSWNSGALTSGVHTFPAVLQSSGLYSLSSVVTVPSSSLGTQTYICNVNHKPSNTKVDKKVEPKSCDKTHTSPPSPAPPVAGPSVFLFPPKPKDTLMISRTPEVTCVVVGVSHEDPEVKFNWYVDGVEVHNAKTKPREEQYQSTYRVVSVLTVLHQDWLNGKEYKCKVSNKQLPSPIEKTISKAKGQPSGEVQLVESGGGLVQPGGSLRLSCAASGYSFTGYTMNWVRQAPGKGLEWVALINPYKGVSTYNQKFKDRFTISVDKSKNTAYLQMNSLRAEDTAVYYCARSGYYGDSDWYFDVWGQGTLVTVSS

SEQ ID NO: 24 - protein, 457 aa, Artificial Sequence
  FLT3 x CD3 Fabv
QVQLKQSGPGLVQPSQSLSITCTVSGFSLTNYGLHWVRQSPGKGLEWLGVIWSGGSTDYNAAFISRLSISKDNSKSQVFFKMNSLQADDTAIYYCARKGGIYYANHYYAMDYWGQGTSVTVSSASTKGPSVFPLAPSSKSTSGGTAALGCLVKDYFPEPVTVSWNSGALTSGVHTFPAVLQSSGLYSLSSVVTVPSSSLGTQTYICNVNHKPSNTKVDKKVEPKSCDKTHTSPPSPAPPVAGPSVFLFPPKPKDTLMISRTPEVTCVVVGVSHEDPEVKFNWYVDGVEVHNAKTKPREEQYQSTYRVVSVLTVLHQDWLNGKEYKCKVSNKQLPSPIEKTISKAKGQPSGDIQMTQSPSSLSASVGDRVTITCRASQDIRNYLNWYQQKPGKAPKLLIYYTSRLESGVPSRFSGSGSGTDYTLTISSLQPEDFATYYCQQGNTLPWTFGQGTKVEIK

SEQ ID NO: 25 - protein, 472 aa, Artificial Sequence
  FLT3 x CD3 Fabv
QVQLKQSGPGLVQPSQSLSITCTVSGFSLTNYGLHWVRQSPGKGLEWLGVIWSGGSTDYNAAFISRLSISKDNSKSQVFFKMNSLQADDTAIYYCARKGGIYYANHYYAMDYWGQGTSVTVSSASTKGPSVFPLAPSSKSTSGGTAALGCLVKDYFPEPVTVSWNSGALTSGVHTFPAVLQSSGLYSLSSVVTVPSSSLGTQTYICNVNHKPSNTKVDKKVEPKSCDKTHTSPPSPAPPVAGPSVFLFPPKPKDTLMISRTPEVTCVVVGVSHEDPEVKFNWYVDGVEVHNAKTKPREEQYQSTYRVVSVLTVLHQDWLNGKEYKCKVSNKQLPSPIEKTISKAKGQPSGEVQLVESGGGLVQPGGSLRLSCAASGYSFTGYTMNWVRQAPGKGLEWVALINPYKGVSTYNQKFKDRFTISVDKSKNTAYLQMNSLRAEDTAVYYCARSGYYGDSDWYFDVWGQGTLVTVSS

SEQ ID NO: 26 - protein, 464 aa, Artificial Sequence
  FLT3 x TCR Fabv
QVQLQQPGAELVKPGASLKLSCKSSGYTFTSYWMHWVRQRPGHGLEWIGEIDPSDSYKDYNQKFKDKATLTVDRSSNTAYMHLSSLTSDDSAVYYCARAITTTPFDFWGQGTTLTVSSASTKGPSVFPLAPSSKSTSGGTAALGCLVKDYFPEPVTVSWNSGALTSGVHTFPAVLQSSGLYSLSSVVTVPSSSLGTQTYICNVNHKPSNTKVDKKVEPKSCDKTHTSPPSPAPPVAGPSVFLFPPKPKDTLMISRTPEVTCVVVGVSHEDPEVKFNWYVDGVEVHNAKTKPREEQYQSTYRVVSVLTVLHQDWLNGKEYKCKVSNKQLPSPIEKTISKAKGQPSGEVQLQQSGPELVKPGASVKMSCKASGYKFTSYVMHWVKQKPGQGLEWIGYINPYNDVTKYNEKFKGKATLTSDKSSSTAYMELSSLTSEDSAVHYCARGSYYDYDGFVYGQGTLVTVSS

SEQ ID NO: 27 - protein, 451 aa, Artificial Sequence
  FLT3 x TCR Fabv
QVQLQQPGAELVKPGASLKLSCKSSGYTFTSYWMHWVRQRPGHGLEWIGEIDPSDSYKDYNQKFKDKATLTVDRSSNTAYMHLSSLTSDDSAVYYCARAITTTPFDFWGQGTTLTVSSASTKGPSVFPLAPSSKSTSGGTAALGCLVKDYFPEPVTVSWNSGALTSGVHTFPAVLQSSGLYSLSSVVTVPSSSLGTQTYICNVNHKPSNTKVDKKVEPKSCDKTHTSPPSPAPPVAGPSVFLFPPKPKDTLMISRTPEVTCVVVGVSHEDPEVKFNWYVDGVEVHNAKTKPREEQYQSTYRVVSVLTVLHQDWLNGKEYKCKVSNKQLPSPIEKTISKAKGQPSGQIVLTQSPAIMSASPGEKVTMTCSATSSVSYMHWYQQKSGTSPKRWIYDTSKLASGVPARFSGSGSGTSYSLTISSMEAEDAATYYCQQWSSNPLTFGAGTKLELK

SEQ ID NO: 28 - protein, 469 aa, Artificial Sequence
  FLT3 x TCR Fabv
QVQLKQSGPGLVQPSQSLSITCTVSGFSLTNYGLHWVRQSPGKGLEWLGVIWSGGSTDYNAAFISRLSISKDNSKSQVFFKMNSLQADDTAIYYCARKGGIYYANHYYAMDYWGQGTSVTVSSASTKGPSVFPLAPSSKSTSGGTAALGCLVKDYFPEPVTVSWNSGALTSGVHTFPAVLQSSGLYSLSSVVTVPSSSLGTQTYICNVNHKPSNTKVDKKVEPKSCDKTHTSPPSPAPPVAGPSVFLFPPKPKDTLMISRTPEVTCVVVGVSHEDPEVKFNWYVDGVEVHNAKTKPREEQYQSTYRVVSVLTVLHQDWLNGKEYKCKVSNKQLPSPIEKTISKAKGQPSGEVQLQQSGPELVKPGASVKMSCKASGYKFTSYVMHWVKQKPGQGLEWIGYINPYNDVTKYNEKFKGKATLTSDKSSSTAYMELSSLTSEDSAVHYCARGSYYDYDGFVYGQGTLVTVSS

SEQ ID NO: 29 - protein, 456 aa, Artificial Sequence
  FLT3 x TCR Fabv
QVQLKQSGPGLVQPSQSLSITCTVSGFSLTNYGLHWVRQSPGKGLEWLGVIWSGGSTDYNAAFISRLSISKDNSKSQVFFKMNSLQADDTAIYYCARKGGIYYANHYYAMDYWGQGTSVTVSSASTKGPSVFPLAPSSKSTSGGTAALGCLVKDYFPEPVTVSWNSGALTSGVHTFPAVLQSSGLYSLSSVVTVPSSSLGTQTYICNVNHKPSNTKVDKKVEPKSCDKTHTSPPSPAPPVAGPSVFLFPPKPKDTLMISRTPEVTCVVVGVSHEDPEVKFNWYVDGVEVHNAKTKPREEQYQSTYRVVSVLTVLHQDWLNGKEYKCKVSNKQLPSPIEKTISKAKGQPSGQIVLTQSPAIMSASPGEKVTMTCSATSSVSYMHWYQQKSGTSPKRWIYDTSKLASGVPARFSGSGSGTSYSLTISSMEAEDAATYYCQQWSSNPLTFGAGTKLELK

SEQ ID NO: 30 - protein, 457 aa, Artificial Sequence
  FLT3 x CD28 Fabv
QVQLQQPGAELVKPGASLKLSCKSSGYTFTSYWMHWVRQRPGHGLEWIGEIDPSDSYKDYNQKFKDKATLTVDRSSNTAYMHLSSLTSDDSAVYYCARAITTTPFDFWGQGTTLTVSSASTKGPSVFPLAPSSKSTSGGTAALGCLVKDYFPEPVTVSWNSGALTSGVHTFPAVLQSSGLYSLSSVVTVPSSSLGTQTYICNVNHKPSNTKVDKKVEPKSCDKTHTSPPSPAPPVAGPSVFLFPPKPKDTLMISRTPEVTCVVVGVSHEDPEVKFNWYVDGVEVHNAKTKPREEQYQSTYRVVSVLTVLHQDWLNGKEYKCKVSNKQLPSPIEKTISKAKGQPSGDIELTQSPASLAVSLGQRATISCRASESVEYYVTSLMQWYQQKPGQPPKLLIFAASNVESGVPARFSGSGSGTNFSLNIHPVDEDDVAMYFCQQSRKVPYTFGGGTKLEIKR

SEQ ID NO: 31 - protein, 465 aa, Artificial Sequence
  FLT3 x CD28 Fabv
QVQLQQPGAELVKPGASLKLSCKSSGYTFTSYWMHWVRQRPGHGLEWIGEIDPSDSYKDYNQKFKDKATLTVDRSSNTAYMHLSSLTSDDSAVYYCARAITTTPFDFWGQGTTLTVSSASTKGPSVFPLAPSSKSTSGGTAALGCLVKDYFPEPVTVSWNSGALTSGVHTFPAVLQSSGLYSLSSVVTVPSSSLGTQTYICNVNHKPSNTKVDKKVEPKSCDKTHTSPPSPAPPVAGPSVFLFPPKPKDTLMISRTPEVTCVVVGVSHEDPEVKFNWYVDGVEVHNAKTKPREEQYQSTYRVVSVLTVLHQDWLNGKEYKCKVSNKQLPSPIEKTISKAKGQPSGQVKLQQSGPGLVTPSQSLSITCTVSGFSLSDYGVHWVRQSPGQGLEWLGVIWAGGGTNYNSALMSRKSISKDNSKSQVFLKMNSLQADDTAVYYCARDKGYSYYYSMDYWGQGTTVTVSS

SEQ ID NO: 32 - protein, 462 aa, Artificial Sequence
  FLT3 x CD28 Fabv
QVQLKQSGPGLVQPSQSLSITCTVSGFSLTNYGLHWVRQSPGKGLEWLGVIWSGGSTDYNAAFISRLSISKDNSKSQVFFKMNSLQADDTAIYYCARKGGIYYANHYYAMDYWGQGTSVTVSSASTKGPSVFPLAPSSKSTSGGTAALGCLVKDYFPEPVTVSWNSGALTSGVHTFPAVLQSSGLYSLSSVVTVPSSSLGTQTYICNVNHKPSNTKVDKKVEPKSCDKTHTSPPSPAPPVAGPSVFLFPPKPKDTLMISRTPEVTCVVVGVSHEDPEVKFNWYVDGVEVHNAKTKPREEQYQSTYRVVSVLTVLHQDWLNGKEYKCKVSNKQLPSPIEKTISKAKGQPSGDIELTQSPASLAVSLGQRATISCRASESVEYYVTSLMQWYQQKPGQPPKLLIFAASNVESGVPARFSGSGSGTNFSLNIHPVDEDDVAMYFCQQSRKVPYTFGGGTKLEIKR

SEQ ID NO: 33 - protein, 470 aa, Artificial Sequence
  FLT3 x CD28 Fabv
QVQLKQSGPGLVQPSQSLSITCTVSGFSLTNYGLHWVRQSPGKGLEWLGVIWSGGSTDYNAAFISRLSISKDNSKSQVFFKMNSLQADDTAIYYCARKGGIYYANHYYAMDYWGQGTSVTVSSASTKGPSVFPLAPSSKSTSGGTAALGCLVKDYFPEPVTVSWNSGALTSGVHTFPAVLQSSGLYSLSSVVTVPSSSLGTQTYICNVNHKPSNTKVDKKVEPKSCDKTHTSPPSPAPPVAGPSVFLFPPKPKDTLMISRTPEVTCVVVGVSHEDPEVKFNWYVDGVEVHNAKTKPREEQYQSTYRVVSVLTVLHQDWLNGKEYKCKVSNKQLPSPIEKTISKAKGQPSGQVKLQQSGPGLVTPSQSLSITCTVSGFSLSDYGVHWVRQSPGQGLEWLGVIWAGGGTNYNSALMSRKSISKDNSKSQVFLKMNSLQADDTAVYYCARDKGYSYYYSMDYWGQGTTVTVSS

SEQ ID NO: 34 - protein, 456 aa, Artificial Sequence
  FLT3 x CD16 Fabv
QVQLQQPGAELVKPGASLKLSCKSSGYTFTSYWMHWVRQRPGHGLEWIGEIDPSDSYKDYNQKFKDKATLTVDRSSNTAYMHLSSLTSDDSAVYYCARAITTTPFDFWGQGTTLTVSSASTKGPSVFPLAPSSKSTSGGTAALGCLVKDYFPEPVTVSWNSGALTSGVHTFPAVLQSSGLYSLSSVVTVPSSSLGTQTYICNVNHKPSNTKVDKKVEPKSCDKTHTSPPSPAPPVAGPSVFLFPPKPKDTLMISRTPEVTCVVVGVSHEDPEVKFNWYVDGVEVHNAKTKPREEQYQSTYRVVSVLTVLHQDWLNGKEYKCKVSNKQLPSPIEKTISKAKGQPSGDIVLTQSPASLAVSLGQRATISCKASQSVDFDGDSFMNWYQQKPGQPPKLLIYTTSNLESGIPARFSASGSGTDFTLNIHPVEEEDTATYYCQQSNEDPYTFGGGTKLEIK

SEQ ID NO: 35 - protein, 463 aa, Artificial Sequence
  FLT3 x CD16 Fabv
QVQLQQPGAELVKPGASLKLSCKSSGYTFTSYWMHWVRQRPGHGLEWIGEIDPSDSYKDYNQKFKDKATLTVDRSSNTAYMHLSSLTSDDSAVYYCARAITTTPFDFWGQGTTLTVSSASTKGPSVFPLAPSSKSTSGGTAALGCLVKDYFPEPVTVSWNSGALTSGVHTFPAVLQSSGLYSLSSVVTVPSSSLGTQTYICNVNHKPSNTKVDKKVEPKSCDKTHTSPPSPAPPVAGPSVFLFPPKPKDTLMISRTPEVTCVVVGVSHEDPEVKFNWYVDGVEVHNAKTKPREEQYQSTYRVVSVLTVLHQDWLNGKEYKCKVSNKQLPSPIEKTISKAKGQPSGQVTLKESGPGILQPSQTLSLTCSFSGFSLRTSGMGVGWIRQPSGKGLEWLAHIWWDDDKRYNPALKSRLTISKDTSSNQVFLKIASVDTADTATYYCAQINPAWFAYWGQGTLVTVSS

SEQ ID NO: 36 - protein, 461 aa, Artificial Sequence
  FLT3 x CD16 Fabv
QVQLKQSGPGLVQPSQSLSITCTVSGFSLTNYGLHWVRQSPGKGLEWLGVIWSGGSTDYNAAFISRLSISKDNSKSQVFFKMNSLQADDTAIYYCARKGGIYYANHYYAMDYWGQGTSVTVSSASTKGPSVFPLAPSSKSTSGGTAALGCLVKDYFPEPVTVSWNSGALTSGVHTFPAVLQSSGLYSLSSVVTVPSSSLGTQTYICNVNHKPSNTKVDKKVEPKSCDKTHTSPPSPAPPVAGPSVFLFPPKPKDTLMISRTPEVTCVVVGVSHEDPEVKFNWYVDGVEVHNAKTKPREEQYQSTYRVVSVLTVLHQDWLNGKEYKCKVSNKQLPSPIEKTISKAKGQPSGDIVLTQSPASLAVSLGQRATISCKASQSVDFDGDSFMNWYQQKPGQPPKLLIYTTSNLESGIPARFSASGSGTDFTLNIHPVEEEDTATYYCQQSNEDPYTFGGGTKLEIK

SEQ ID NO: 37 - protein, 468 aa, Artificial Sequence
  FLT3 x CD16 Fabv
QVQLKQSGPGLVQPSQSLSITCTVSGFSLTNYGLHWVRQSPGKGLEWLGVIWSGGSTDYNAAFISRLSISKDNSKSQVFFKMNSLQADDTAIYYCARKGGIYYANHYYAMDYWGQGTSVTVSSASTKGPSVFPLAPSSKSTSGGTAALGCLVKDYFPEPVTVSWNSGALTSGVHTFPAVLQSSGLYSLSSVVTVPSSSLGTQTYICNVNHKPSNTKVDKKVEPKSCDKTHTSPPSPAPPVAGPSVFLFPPKPKDTLMISRTPEVTCVVVGVSHEDPEVKFNWYVDGVEVHNAKTKPREEQYQSTYRVVSVLTVLHQDWLNGKEYKCKVSNKQLPSPIEKTISKAKGQPSGQVTLKESGPGILQPSQTLSLTCSFSGFSLRTSGMGVGWIRQPSGKGLEWLAHIWWDDDKRYNPALKSRLTISKDTSSNQVFLKIASVDTADTATYYCAQINPAWFAYWGQGTLVTVSS

SEQ ID NO: 38 - protein, 455 aa, Artificial Sequence
  CD19 x CD3 Fabv
EVQLQQSGPELIKPGASVKMSCKASGYTFTSYVMHWVKQKPGQGLEWIGYINPYNDGTKYNEKFKGKATLTSDKSSSTAYMELSSLTSEDSAVYYCARGTYYYGSRVFDYWGQGTTLTVSSASTKGPSVFPLAPSSKSTSGGTAALGCLVKDYFPEPVTVSWNSGALTSGVHTFPAVLQSSGLYSLSSVVTVPSSSLGTQTYICNVNHKPSNTKVDKKVEPKSCDKTHTSPPSPAPPVAGPSVFLFPPKPKDTLMISRTPEVTCVVVGVSHEDPEVKFNWYVDGVEVHNAKTKPREEQYQSTYRVVSVLTVLHQDWLNGKEYKCKVSNKQLPSPIEKTISKAKGQPSGDIQMTQSPSSLSASVGDRVTITCRASQDIRNYLNWYQQKPGKAPKLLIYYTSRLESGVPSRFSGSGSGTDYTLTISSLQPEDFATYYCQQGNTLPWTFGQGTKVEIK

SEQ ID NO: 39 - protein, 470 aa, Artificial Sequence
  CD19 x CD3 Fabv
EVQLQQSGPELIKPGASVKMSCKASGYTFTSYVMHWVKQKPGQGLEWIGYINPYNDGTKYNEKFKGKATLTSDKSSSTAYMELSSLTSEDSAVYYCARGTYYYGSRVFDYWGQGTTLTVSSASTKGPSVFPLAPSSKSTSGGTAALGCLVKDYFPEPVTVSWNSGALTSGVHTFPAVLQSSGLYSLSSVVTVPSSSLGTQTYICNVNHKPSNTKVDKKVEPKSCDKTHTSPPSPAPPVAGPSVFLFPPKPKDTLMISRTPEVTCVVVGVSHEDPEVKFNWYVDGVEVHNAKTKPREEQYQSTYRVVSVLTVLHQDWLNGKEYKCKVSNKQLPSPIEKTISKAKGQPSGEVQLVESGGGLVQPGGSLRLSCAASGYSFTGYTMNWVRQAPGKGLEWVALINPYKGVSTYNQKFKDRFTISVDKSKNTAYLQMNSLRAEDTAVYYCARSGYYGDSDWYFDVWGQGTLVTVSS

SEQ ID NO: 40 - protein, 467 aa, Artificial Sequence
  CD19 x TCR Fabv
EVQLQQSGPELIKPGASVKMSCKASGYTFTSYVMHWVKQKPGQGLEWIGYINPYNDGTKYNEKFKGKATLTSDKSSSTAYMELSSLTSEDSAVYYCARGTYYYGSRVFDYWGQGTTLTVSSASTKGPSVFPLAPSSKSTSGGTAALGCLVKDYFPEPVTVSWNSGALTSGVHTFPAVLQSSGLYSLSSVVTVPSSSLGTQTYICNVNHKPSNTKVDKKVEPKSCDKTHTSPPSPAPPVAGPSVFLFPPKPKDTLMISRTPEVTCVVVGVSHEDPEVKFNWYVDGVEVHNAKTKPREEQYQSTYRVVSVLTVLHQDWLNGKEYKCKVSNKQLPSPIEKTISKAKGQPSGEVQLQQSGPELVKPGASVKMSCKASGYKFTSYVMHWVKQKPGQGLEWIGYINPYNDVTKYNEKFKGKATLTSDKSSSTAYMELSSLTSEDSAVHYCARGSYYDYDGFVYGQGTLVTVSS

SEQ ID NO: 41 - protein, 454 aa, Artificial Sequence
  CD19 x TCR Fabv
EVQLQQSGPELIKPGASVKMSCKASGYTFTSYVMHWVKQKPGQGLEWIGYINPYNDGTKYNEKFKGKATLTSDKSSSTAYMELSSLTSEDSAVYYCARGTYYYGSRVFDYWGQGTTLTVSSASTKGPSVFPLAPSSKSTSGGTAALGCLVKDYFPEPVTVSWNSGALTSGVHTFPAVLQSSGLYSLSSVVTVPSSSLGTQTYICNVNHKPSNTKVDKKVEPKSCDKTHTSPPSPAPPVAGPSVFLFPPKPKDTLMISRTPEVTCVVVGVSHEDPEVKFNWYVDGVEVHNAKTKPREEQYQSTYRVVSVLTVLHQDWLNGKEYKCKVSNKQLPSPIEKTISKAKGQPSGQIVLTQSPAIMSASPGEKVTMTCSATSSVSYMHWYQQKSGTSPKRWIYDTSKLASGVPARFSGSGSGTSYSLTISSMEAEDAATYYCQQWSSNPLTFGAGTKLELK

SEQ ID NO: 42 - protein, 460 aa, Artificial Sequence
  CD19 x CD28 Fabv
EVQLQQSGPELIKPGASVKMSCKASGYTFTSYVMHWVKQKPGQGLEWIGYINPYNDGTKYNEKFKGKATLTSDKSSSTAYMELSSLTSEDSAVYYCARGTYYYGSRVFDYWGQGTTLTVSSASTKGPSVFPLAPSSKSTSGGTAALGCLVKDYFPEPVTVSWNSGALTSGVHTFPAVLQSSGLYSLSSVVTVPSSSLGTQTYICNVNHKPSNTKVDKKVEPKSCDKTHTSPPSPAPPVAGPSVFLFPPKPKDTLMISRTPEVTCVVVGVSHEDPEVKFNWYVDGVEVHNAKTKPREEQYQSTYRVVSVLTVLHQDWLNGKEYKCKVSNKQLPSPIEKTISKAKGQPSGDIELTQSPASLAVSLGQRATISCRASESVEYYVTSLMQWYQQKPGQPPKLLIFAASNVESGVPARFSGSGSGTNFSLNIHPVDEDDVAMYFCQQSRKVPYTFGGGTKLEIKR

SEQ ID NO: 43 - protein, 468 aa, Artificial Sequence
  CD19 x CD28 Fabv
EVQLQQSGPELIKPGASVKMSCKASGYTFTSYVMHWVKQKPGQGLEWIGYINPYNDGTKYNEKFKGKATLTSDKSSSTAYMELSSLTSEDSAVYYCARGTYYYGSRVFDYWGQGTTLTVSSASTKGPSVFPLAPSSKSTSGGTAALGCLVKDYFPEPVTVSWNSGALTSGVHTFPAVLQSSGLYSLSSVVTVPSSSLGTQTYICNVNHKPSNTKVDKKVEPKSCDKTHTSPPSPAPPVAGPSVFLFPPKPKDTLMISRTPEVTCVVVGVSHEDPEVKFNWYVDGVEVHNAKTKPREEQYQSTYRVVSVLTVLHQDWLNGKEYKCKVSNKQLPSPIEKTISKAKGQPSGQVKLQQSGPGLVTPSQSLSITCTVSGFSLSDYGVHWVRQSPGQGLEWLGVIWAGGGTNYNSALMSRKSISKDNSKSQVFLKMNSLQADDTAVYYCARDKGYSYYYSMDYWGQGTTVTVSS

SEQ ID NO: 44 - protein, 459 aa, Artificial Sequence
  CD19 x CD16 Fabv
EVQLQQSGPELIKPGASVKMSCKASGYTFTSYVMHWVKQKPGQGLEWIGYINPYNDGTKYNEKFKGKATLTSDKSSSTAYMELSSLTSEDSAVYYCARGTYYYGSRVFDYWGQGTTLTVSSASTKGPSVFPLAPSSKSTSGGTAALGCLVKDYFPEPVTVSWNSGALTSGVHTFPAVLQSSGLYSLSSVVTVPSSSLGTQTYICNVNHKPSNTKVDKKVEPKSCDKTHTSPPSPAPPVAGPSVFLFPPKPKDTLMISRTPEVTCVVVGVSHEDPEVKFNWYVDGVEVHNAKTKPREEQYQSTYRVVSVLTVLHQDWLNGKEYKCKVSNKQLPSPIEKTISKAKGQPSGDIVLTQSPASLAVSLGQRATISCKASQSVDFDGDSFMNWYQQKPGQPPKLLIYTTSNLESGIPARFSASGSGTDFTLNIHPVEEEDTATYYCQQSNEDPYTFGGGTKLEIK

SEQ ID NO: 45 - protein, 466 aa, Artificial Sequence
  CD19 x CD16 Fabv
EVQLQQSGPELIKPGASVKMSCKASGYTFTSYVMHWVKQKPGQGLEWIGYINPYNDGTKYNEKFKGKATLTSDKSSSTAYMELSSLTSEDSAVYYCARGTYYYGSRVFDYWGQGTTLTVSSASTKGPSVFPLAPSSKSTSGGTAALGCLVKDYFPEPVTVSWNSGALTSGVHTFPAVLQSSGLYSLSSVVTVPSSSLGTQTYICNVNHKPSNTKVDKKVEPKSCDKTHTSPPSPAPPVAGPSVFLFPPKPKDTLMISRTPEVTCVVVGVSHEDPEVKFNWYVDGVEVHNAKTKPREEQYQSTYRVVSVLTVLHQDWLNGKEYKCKVSNKQLPSPIEKTISKAKGQPSGQVTLKESGPGILQPSQTLSLTCSFSGFSLRTSGMGVGWIRQPSGKGLEWLAHIWWDDDKRYNPALKSRLTISKDTSSNQVFLKIASVDTADTATYYCAQINPAWFAYWGQGTLVTVSS

SEQ ID NO: 46 - protein, 455 aa, Artificial Sequence
  CSPG4 x CD3 Fabv
QVKLQQSGPELVKPGASVKISCKASGYAFSRSWMNWVKQRPGQGLEWIGRIYPGDGDTNYNGKFKGKATLTADKSSSTAYMQVSSLTSVDSAVYFCARGNTVVVPYTMDYWGQGTTVTVSSASTKGPSVFPLAPSSKSTSGGTAALGCLVKDYFPEPVTVSWNSGALTSGVHTFPAVLQSSGLYSLSSVVTVPSSSLGTQTYICNVNHKPSNTKVDKKVEPKSCDKTHTSPPSPAPPVAGPSVFLFPPKPKDTLMISRTPEVTCVVVGVSHEDPEVKFNWYVDGVEVHNAKTKPREEQYQSTYRVVSVLTVLHQDWLNGKEYKCKVSNKQLPSPIEKTISKAKGQPSGDIQMTQSPSSLSASVGDRVTITCRASQDIRNYLNWYQQKPGKAPKLLIYYTSRLESGVPSRFSGSGSGTDYTLTISSLQPEDFATYYCQQGNTLPWTFGQGTKVEIK

SEQ ID NO: 47 - protein, 470 aa, Artificial Sequence
  CSPG4 x CD3 Fabv
QVKLQQSGPELVKPGASVKISCKASGYAFSRSWMNWVKQRPGQGLEWIGRIYPGDGDTNYNGKFKGKATLTADKSSSTAYMQVSSLTSVDSAVYFCARGNTVVVPYTMDYWGQGTTVTVSSASTKGPSVFPLAPSSKSTSGGTAALGCLVKDYFPEPVTVSWNSGALTSGVHTFPAVLQSSGLYSLSSVVTVPSSSLGTQTYICNVNHKPSNTKVDKKVEPKSCDKTHTSPPSPAPPVAGPSVFLFPPKPKDTLMISRTPEVTCVVVGVSHEDPEVKFNWYVDGVEVHNAKTKPREEQYQSTYRVVSVLTVLHQDWLNGKEYKCKVSNKQLPSPIEKTISKAKGQPSGEVQLVESGGGLVQPGGSLRLSCAASGYSFTGYTMNWVRQAPGKGLEWVALINPYKGVSTYNQKFKDRFTISVDKSKNTAYLQMNSLRAEDTAVYYCARSGYYGDSDWYFDVWGQGTLVTVSS

SEQ ID NO: 48 - protein, 467 aa, Artificial Sequence
  CSPG4 x TCR Fabv
QVKLQQSGPELVKPGASVKISCKASGYAFSRSWMNWVKQRPGQGLEWIGRIYPGDGDTNYNGKFKGKATLTADKSSSTAYMQVSSLTSVDSAVYFCARGNTVVVPYTMDYWGQGTTVTVSSASTKGPSVFPLAPSSKSTSGGTAALGCLVKDYFPEPVTVSWNSGALTSGVHTFPAVLQSSGLYSLSSVVTVPSSSLGTQTYICNVNHKPSNTKVDKKVEPKSCDKTHTSPPSPAPPVAGPSVFLFPPKPKDTLMISRTPEVTCVVVGVSHEDPEVKFNWYVDGVEVHNAKTKPREEQYQSTYRVVSVLTVLHQDWLNGKEYKCKVSNKQLPSPIEKTISKAKGQPSGEVQLQQSGPELVKPGASVKMSCKASGYKFTSYVMHWVKQKPGQGLEWIGYINPYNDVTKYNEKFKGKATLTSDKSSSTAYMELSSLTSEDSAVHYCARGSYYDYDGFVYGQGTLVTVSS

SEQ ID NO: 49 - protein, 454 aa, Artificial Sequence
  CSPG4 x TCR Fabv
QVKLQQSGPELVKPGASVKISCKASGYAFSRSWMNWVKQRPGQGLEWIGRIYPGDGDTNYNGKFKGKATLTADKSSSTAYMQVSSLTSVDSAVYFCARGNTVVVPYTMDYWGQGTTVTVSSASTKGPSVFPLAPSSKSTSGGTAALGCLVKDYFPEPVTVSWNSGALTSGVHTFPAVLQSSGLYSLSSVVTVPSSSLGTQTYICNVNHKPSNTKVDKKVEPKSCDKTHTSPPSPAPPVAGPSVFLFPPKPKDTLMISRTPEVTCVVVGVSHEDPEVKFNWYVDGVEVHNAKTKPREEQYQSTYRVVSVLTVLHQDWLNGKEYKCKVSNKQLPSPIEKTISKAKGQPSGQIVLTQSPAIMSASPGEKVTMTCSATSSVSYMHWYQQKSGTSPKRWIYDTSKLASGVPARFSGSGSGTSYSLTISSMEAEDAATYYCQQWSSNPLTFGAGTKLELK

SEQ ID NO: 50 - protein, 460 aa, Artificial Sequence
  CSPG4 x CD28 Fabv
QVKLQQSGPELVKPGASVKISCKASGYAFSRSWMNWVKQRPGQGLEWIGRIYPGDGDTNYNGKFKGKATLTADKSSSTAYMQVSSLTSVDSAVYFCARGNTVVVPYTMDYWGQGTTVTVSSASTKGPSVFPLAPSSKSTSGGTAALGCLVKDYFPEPVTVSWNSGALTSGVHTFPAVLQSSGLYSLSSVVTVPSSSLGTQTYICNVNHKPSNTKVDKKVEPKSCDKTHTSPPSPAPPVAGPSVFLFPPKPKDTLMISRTPEVTCVVVGVSHEDPEVKFNWYVDGVEVHNAKTKPREEQYQSTYRVVSVLTVLHQDWLNGKEYKCKVSNKQLPSPIEKTISKAKGQPSGDIELTQSPASLAVSLGQRATISCRASESVEYYVTSLMQWYQQKPGQPPKLLIFAASNVESGVPARFSGSGSGTNFSLNIHPVDEDDVAMYFCQQSRKVPYTFGGGTKLEIKR

SEQ ID NO: 51 - protein, 468 aa, Artificial Sequence
  CSPG4 x CD28 Fabv
QVKLQQSGPELVKPGASVKISCKASGYAFSRSWMNWVKQRPGQGLEWIGRIYPGDGDTNYNGKFKGKATLTADKSSSTAYMQVSSLTSVDSAVYFCARGNTVVVPYTMDYWGQGTTVTVSSASTKGPSVFPLAPSSKSTSGGTAALGCLVKDYFPEPVTVSWNSGALTSGVHTFPAVLQSSGLYSLSSVVTVPSSSLGTQTYICNVNHKPSNTKVDKKVEPKSCDKTHTSPPSPAPPVAGPSVFLFPPKPKDTLMISRTPEVTCVVVGVSHEDPEVKFNWYVDGVEVHNAKTKPREEQYQSTYRVVSVLTVLHQDWLNGKEYKCKVSNKQLPSPIEKTISKAKGQPSGQVKLQQSGPGLVTPSQSLSITCTVSGFSLSDYGVHWVRQSPGQGLEWLGVIWAGGGTNYNSALMSRKSISKDNSKSQVFLKMNSLQADDTAVYYCARDKGYSYYYSMDYWGQGTTVTVSS

SEQ ID NO: 52 - protein, 459 aa, Artificial Sequence
  CSPG4 x CD16 Fabv
QVKLQQSGPELVKPGASVKISCKASGYAFSRSWMNWVKQRPGQGLEWIGRIYPGDGDTNYNGKFKGKATLTADKSSSTAYMQVSSLTSVDSAVYFCARGNTVVVPYTMDYWGQGTTVTVSSASTKGPSVFPLAPSSKSTSGGTAALGCLVKDYFPEPVTVSWNSGALTSGVHTFPAVLQSSGLYSLSSVVTVPSSSLGTQTYICNVNHKPSNTKVDKKVEPKSCDKTHTSPPSPAPPVAGPSVFLFPPKPKDTLMISRTPEVTCVVVGVSHEDPEVKFNWYVDGVEVHNAKTKPREEQYQSTYRVVSVLTVLHQDWLNGKEYKCKVSNKQLPSPIEKTISKAKGQPSGDIVLTQSPASLAVSLGQRATISCKASQSVDFDGDSFMNWYQQKPGQPPKLLIYTTSNLESGIPARFSASGSGTDFTLNIHPVEEEDTATYYCQQSNEDPYTFGGGTKLEIK

SEQ ID NO: 53 - protein, 466 aa, Artificial Sequence
  CSPG4 x CD16 Fabv
QVKLQQSGPELVKPGASVKISCKASGYAFSRSWMNWVKQRPGQGLEWIGRIYPGDGDTNYNGKFKGKATLTADKSSSTAYMQVSSLTSVDSAVYFCARGNTVVVPYTMDYWGQGTTVTVSSASTKGPSVFPLAPSSKSTSGGTAALGCLVKDYFPEPVTVSWNSGALTSGVHTFPAVLQSSGLYSLSSVVTVPSSSLGTQTYICNVNHKPSNTKVDKKVEPKSCDKTHTSPPSPAPPVAGPSVFLFPPKPKDTLMISRTPEVTCVVVGVSHEDPEVKFNWYVDGVEVHNAKTKPREEQYQSTYRVVSVLTVLHQDWLNGKEYKCKVSNKQLPSPIEKTISKAKGQPSGQVTLKESGPGILQPSQTLSLTCSFSGFSLRTSGMGVGWIRQPSGKGLEWLAHIWWDDDKRYNPALKSRLTISKDTSSNQVFLKIASVDTADTATYYCAQINPAWFAYWGQGTLVTVSS

SEQ ID NO: 54 - protein, 453 aa, Artificial Sequence
  EGFR x CD3 Fabv
QVQLKQSGPGLVQPSQSLSITCTVSGFSLTNYGVHWVRQSPGKGLEWLGVIWSGGNTDYNTPFTSRLSINKDNSKSQVFFKMNSLQSNDTAIYYCARALTYYDYEFAYWGQGTLVTVSSASTKGPSVFPLAPSSKSTSGGTAALGCLVKDYFPEPVTVSWNSGALTSGVHTFPAVLQSSGLYSLSSVVTVPSSSLGTQTYICNVNHKPSNTKVDKKVEPKSCDKTHTSPPSPAPPVAGPSVFLFPPKPKDTLMISRTPEVTCVVVGVSHEDPEVKFNWYVDGVEVHNAKTKPREEQYQSTYRVVSVLTVLHQDWLNGKEYKCKVSNKQLPSPIEKTISKAKGQPSGDIQMTQSPSSLSASVGDRVTITCRASQDIRNYLNWYQQKPGKAPKLLIYYTSRLESGVPSRFSGSGSGTDYTLTISSLQPEDFATYYCQQGNTLPWTFGQGTKVEIK

SEQ ID NO: 55 - protein, 468 aa, Artificial Sequence
  EGFR x CD3 Fabv
QVQLKQSGPGLVQPSQSLSITCTVSGFSLTNYGVHWVRQSPGKGLEWLGVIWSGGNTDYNTPFTSRLSINKDNSKSQVFFKMNSLQSNDTAIYYCARALTYYDYEFAYWGQGTLVTVSSASTKGPSVFPLAPSSKSTSGGTAALGCLVKDYFPEPVTVSWNSGALTSGVHTFPAVLQSSGLYSLSSVVTVPSSSLGTQTYICNVNHKPSNTKVDKKVEPKSCDKTHTSPPSPAPPVAGPSVFLFPPKPKDTLMISRTPEVTCVVVGVSHEDPEVKFNWYVDGVEVHNAKTKPREEQYQSTYRVVSVLTVLHQDWLNGKEYKCKVSNKQLPSPIEKTISKAKGQPSGEVQLVESGGGLVQPGGSLRLSCAASGYSFTGYTMNWVRQAPGKGLEWVALINPYKGVSTYNQKFKDRFTISVDKSKNTAYLQMNSLRAEDTAVYYCARSGYYGDSDWYFDVWGQGTLVTVSS

SEQ ID NO: 56 - protein, 465 aa, Artificial Sequence
  EGFR x TCR Fabv
QVQLKQSGPGLVQPSQSLSITCTVSGFSLTNYGVHWVRQSPGKGLEWLGVIWSGGNTDYNTPFTSRLSINKDNSKSQVFFKMNSLQSNDTAIYYCARALTYYDYEFAYWGQGTLVTVSSASTKGPSVFPLAPSSKSTSGGTAALGCLVKDYFPEPVTVSWNSGALTSGVHTFPAVLQSSGLYSLSSVVTVPSSSLGTQTYICNVNHKPSNTKVDKKVEPKSCDKTHTSPPSPAPPVAGPSVFLFPPKPKDTLMISRTPEVTCVVVGVSHEDPEVKFNWYVDGVEVHNAKTKPREEQYQSTYRVVSVLTVLHQDWLNGKEYKCKVSNKQLPSPIEKTISKAKGQPSGEVQLQQSGPELVKPGASVKMSCKASGYKFTSYVMHWVKQKPGQGLEWIGYINPYNDVTKYNEKFKGKATLTSDKSSSTAYMELSSLTSEDSAVHYCARGSYYDYDGFVYGQGTLVTVSS

SEQ ID NO: 57 - protein, 452 aa, Artificial Sequence
  EGFR x TCR Fabv
QVQLKQSGPGLVQPSQSLSITCTVSGFSLTNYGVHWVRQSPGKGLEWLGVIWSGGNTDYNTPFTSRLSINKDNSKSQVFFKMNSLQSNDTAIYYCARALTYYDYEFAYWGQGTLVTVSSASTKGPSVFPLAPSSKSTSGGTAALGCLVKDYFPEPVTVSWNSGALTSGVHTFPAVLQSSGLYSLSSVVTVPSSSLGTQTYICNVNHKPSNTKVDKKVEPKSCDKTHTSPPSPAPPVAGPSVFLFPPKPKDTLMISRTPEVTCVVVGVSHEDPEVKFNWYVDGVEVHNAKTKPREEQYQSTYRVVSVLTVLHQDWLNGKEYKCKVSNKQLPSPIEKTISKAKGQPSGQIVLTQSPAIMSASPGEKVTMTCSATSSVSYMHWYQQKSGTSPKRWIYDTSKLASGVPARFSGSGSGTSYSLTISSMEAEDAATYYCQQWSSNPLTFGAGTKLELK

SEQ ID NO: 58 - protein, 458 aa, Artificial Sequence
  EGFR x CD28 Fabv
QVQLKQSGPGLVQPSQSLSITCTVSGFSLTNYGVHWVRQSPGKGLEWLGVIWSGGNTDYNTPFTSRLSINKDNSKSQVFFKMNSLQSNDTAIYYCARALTYYDYEFAYWGQGTLVTVSSASTKGPSVFPLAPSSKSTSGGTAALGCLVKDYFPEPVTVSWNSGALTSGVHTFPAVLQSSGLYSLSSVVTVPSSSLGTQTYICNVNHKPSNTKVDKKVEPKSCDKTHTSPPSPAPPVAGPSVFLFPPKPKDTLMISRTPEVTCVVVGVSHEDPEVKFNWYVDGVEVHNAKTKPREEQYQSTYRVVSVLTVLHQDWLNGKEYKCKVSNKQLPSPIEKTISKAKGQPSGDIELTQSPASLAVSLGQRATISCRASESVEYYVTSLMQWYQQKPGQPPKLLIFAASNVESGVPARFSGSGSGTNFSLNIHPVDEDDVAMYFCQQSRKVPYTFGGGTKLEIKR

SEQ ID NO: 59 - protein, 466 aa, Artificial Sequence
  EGFR x CD28 Fabv
QVQLKQSGPGLVQPSQSLSITCTVSGFSLTNYGVHWVRQSPGKGLEWLGVIWSGGNTDYNTPFTSRLSINKDNSKSQVFFKMNSLQSNDTAIYYCARALTYYDYEFAYWGQGTLVTVSSASTKGPSVFPLAPSSKSTSGGTAALGCLVKDYFPEPVTVSWNSGALTSGVHTFPAVLQSSGLYSLSSVVTVPSSSLGTQTYICNVNHKPSNTKVDKKVEPKSCDKTHTSPPSPAPPVAGPSVFLFPPKPKDTLMISRTPEVTCVVVGVSHEDPEVKFNWYVDGVEVHNAKTKPREEQYQSTYRVVSVLTVLHQDWLNGKEYKCKVSNKQLPSPIEKTISKAKGQPSGQVKLQQSGPGLVTPSQSLSITCTVSGFSLSDYGVHWVRQSPGQGLEWLGVIWAGGGTNYNSALMSRKSISKDNSKSQVFLKMNSLQADDTAVYYCARDKGYSYYYSMDYWGQGTTVTVSS

SEQ ID NO: 60 - protein, 457 aa, Artificial Sequence
  EGFR x CD16 Fabv
QVQLKQSGPGLVQPSQSLSITCTVSGFSLTNYGVHWVRQSPGKGLEWLGVIWSGGNTDYNTPFTSRLSINKDNSKSQVFFKMNSLQSNDTAIYYCARALTYYDYEFAYWGQGTLVTVSSASTKGPSVFPLAPSSKSTSGGTAALGCLVKDYFPEPVTVSWNSGALTSGVHTFPAVLQSSGLYSLSSVVTVPSSSLGTQTYICNVNHKPSNTKVDKKVEPKSCDKTHTSPPSPAPPVAGPSVFLFPPKPKDTLMISRTPEVTCVVVGVSHEDPEVKFNWYVDGVEVHNAKTKPREEQYQSTYRVVSVLTVLHQDWLNGKEYKCKVSNKQLPSPIEKTISKAKGQPSGDIVLTQSPASLAVSLGQRATISCKASQSVDFDGDSFMNWYQQKPGQPPKLLIYTTSNLESGIPARFSASGSGTDFTLNIHPVEEEDTATYYCQQSNEDPYTFGGGTKLEIK

SEQ ID NO: 61 - protein, 464 aa, Artificial Sequence
  EGFR x CD16 Fabv
QVQLKQSGPGLVQPSQSLSITCTVSGFSLTNYGVHWVRQSPGKGLEWLGVIWSGGNTDYNTPFTSRLSINKDNSKSQVFFKMNSLQSNDTAIYYCARALTYYDYEFAYWGQGTLVTVSSASTKGPSVFPLAPSSKSTSGGTAALGCLVKDYFPEPVTVSWNSGALTSGVHTFPAVLQSSGLYSLSSVVTVPSSSLGTQTYICNVNHKPSNTKVDKKVEPKSCDKTHTSPPSPAPPVAGPSVFLFPPKPKDTLMISRTPEVTCVVVGVSHEDPEVKFNWYVDGVEVHNAKTKPREEQYQSTYRVVSVLTVLHQDWLNGKEYKCKVSNKQLPSPIEKTISKAKGQPSGQVTLKESGPGILQPSQTLSLTCSFSGFSLRTSGMGVGWIRQPSGKGLEWLAHIWWDDDKRYNPALKSRLTISKDTSSNQVFLKIASVDTADTATYYCAQINPAWFAYWGQGTLVTVSS

SEQ ID NO: 62 - protein, 106 aa, Artificial Sequence
  CD3 single variable domain (clone OKT3) VL
DIVLTQSPAIMSASPGEKVTMTCSASSSVSYMNWYQQKSGTSPKRWIYDTSKLASGVPAHFRGSGSGTSYSLTISGMEAEDAATYYCQQWSSNPFTFGSGTKLEIN

SEQ ID NO: 63 - protein, 119 aa, Artificial Sequence [sequence omitted]

SEQ ID NO: 64 - DNA, 49 bp, Artificial Sequence
  4G7-H-for
ctcttcacaggtgtcctctctgaggtccagctgcagcagtctggacctg

SEQ ID NO: 65 - DNA, 59 bp, Artificial Sequence
  4G7-H-rev
gggagaaggtaggactcacctgaggagactgtgagagtggtgccttggccccagtagtc

SEQ ID NO: 66 - DNA, 51 bp, Artificial Sequence
  9.2.27-H-for
tcttcacaggtgtcctctcccaggtgaagctgcagcaatctggacctgagc

SEQ ID NO: 67 - DNA, 51 bp, Artificial Sequence
  9.2.27-H-rev
aatgggagaaggtaggactcacctgaggagacggtgaccgtggtcccttgg

SEQ ID NO: 68 - DNA, 53 bp, Artificial Sequence
  4G8-H-for
tctcttcacaggtgtcctctctcaggtccaactgcagcagcctggggctgagc

SEQ ID NO: 69 - DNA, 52 bp, Artificial Sequence
  4G8-H-rev
gagaaggtaggactcacctgaggagactgtgagagtggtgccttggccccag

SEQ ID NO: 70 - DNA, 60 bp, Artificial Sequence
  BV10-H-for
agacgtccactctgtctttctcttcacaggtgtcctctcccaggtgcagctgaagcagtc

SEQ ID NO: 71 - DNA, 49 bp, Artificial Sequence
  BV10-H-rev
gagaaggtaggactcacctgaggagacggtgactgaggttccttgaccc

SEQ ID NO: 72 - DNA, 40 bp, Artificial Sequence
  universal for (AatII)
agacgtccactctgtctttctcttcacaggtgtcctctcc

SEQ ID NO: 73 - DNA, 33 bp, Artificial Sequence
  universal rev (ClaI)
tatcgatttagaatgggagaaggtaggactcac

SEQ ID NO: 74 - DNA, 43 bp, Artificial Sequence
  4G7-L-for (XhoI)
actcgaggagatattgtgatgactcaggctgcaccctctatac

SEQ ID NO: 75 - DNA, 48 bp, Artificial Sequence
  4G7-L-rev (SpeI)
aactagtacttacgtttcagctccagcttggtcccagcaccgaacgtg

SEQ ID NO: 76 - DNA, 42 bp, Artificial Sequence
  9.2.27-L-for (XhoI)
tctcgaggagacatcgagctcactcagtctccagcttctttg

SEQ ID NO: 77 - DNA, 46 bp, Artificial Sequence
  9.2.27-L-rev (SpeI)
aactagtacttacgtttgatctccagcttggtgccccctccaaagg

SEQ ID NO: 78 - DNA, 42 bp, Artificial Sequence
  4G8-L-for (XhoI)
actcgaggagatattgtgctaactcagtctccagccaccctg

SEQ ID NO: 79 - DNA, 41 bp, Artificial Sequence
  4G8-L-rev (SpeI)
tactagtacttacgttttatttccagcttggtcccccctcc

SEQ ID NO: 80 - DNA, 40 bp, Artificial Sequence
  BV10-L-for (XhoI)
actcgaggagacattgtgatgacacagtctccatcctccc

SEQ ID NO: 81 - DNA, 47 bp, Artificial Sequence
  BV10-L-rev (SpeI)
actagtacttacgtttcagctccagcttggtcccagcaccgaacgtg

SEQ ID NO: 82 - DNA, 47 bp, Artificial Sequence
  UCHT1-H-for (BspEI)
ttccggagaggttcagctggtggagtctggcggtggcctggtgcagc

SEQ ID NO: 83 - DNA, 48 bp, Artificial Sequence
  UCHT1-H-rev (SpeI)
tactagttatcacgaggagacggtgaccagggttccttgaccccagac

SEQ ID NO: 84 - DNA, 42 bp, Artificial Sequence
  UCHT1-L-for (BspEI)
ttccggagatatccagatgacccagtccccgagctccctgtc

SEQ ID NO: 85 - DNA, 49 bp, Artificial Sequence
  UCHT1-L-rev (SpeI)
tactagttatcatttgatctccaccttggtgccctgtccgaacgtccac

SEQ ID NO: 86 - DNA, 27 bp, Artificial Sequence
  BMA031-H-for (BspEI)
ttccggagaagtgcagctgcagcagtc

SEQ ID NO: 87 - DNA, 35 bp, Artificial Sequence
  BMA031-H-rev SpeI
tactagttatcagctagacacggtgaccagagtgc

SEQ ID NO: 88 - DNA, 27 bp, Artificial Sequence
  BMA031-L-for (BspEI)
ttccggacagatcgtgctgacccagtc

SEQ ID NO: 89 - DNA, 25 bp, Artificial Sequence
  BMA031-L-rev (SpeI)
tactagttatcacttcagttccagc

SEQ ID NO: 90 - DNA, 26 bp, Artificial Sequence
  OKT3-H-for (BspEI)
ttccggacaggtgcagctgcagcagt

SEQ ID NO: 91 - DNA, 35 bp, Artificial Sequence
  OKT3-H-rev (SpeI)
tactagttatcatgaggagacggtgagcgtggtcc

SEQ ID NO: 92 - DNA, 25 bp, Artificial Sequence
  OKT3-L-for (BspEI)
ttccggagacattgtgctcacccag

SEQ ID NO: 93 - DNA, 32 bp, Artificial Sequence
  OKT3-L-rev (SpeI)
tactagttatcagtttatttccaactttgtcc

SEQ ID NO: 94 - DNA, 47 bp, Artificial Sequence
  9.3-for (BspEI)
ttccggacaggtgaagctgcagcagtctggccctggcctggtgaccc

SEQ ID NO: 95 - DNA, 48 bp, Artificial Sequence
  9.3-H-rev (SpeI)
tactagttatcaagagctcacagtcactgtggtgccctggccccagta

SEQ ID NO: 96 - DNA, 41 bp, Artificial Sequence
  9.3-L-for (BspEI)
ttccggagacattgtgctgacccagtcccctgcctccctgg

SEQ ID NO: 97 - DNA, 49 bp, Artificial Sequence
  9.3-L-rev (SpeI)
tactagttatcacctcttgatctccagcttggtgccccctccaaaggtg

SEQ ID NO: 98 - protein, 11 aa, Artificial Sequence
  parts of the hinge region and CH2 region
SPPSPAPPVAG

SEQ ID NO: 99 - protein, 12 aa, Artificial Sequence
  Parts of the hinge and CH2 region
CPPCPAPELLGG

SEQ ID NO: 100 - protein, 451 aa, Artificial Sequence
  FLT3 x CD3 Fabv
QVQLQQPGAELVKPGASLKLSCKSSGYTFTSYWMHWVRQRPGHGLEWIGEIDPSDSYKDYNQKFKDKATLTVDRSSNTAYMHLSSLTSDDSAVYYCARAITTTPFDFWGQGTTLTVSSASTKGPSVFPLAPSSKSTSGGTAALGCLVKDYFPEPVTVSWNSGALTSGVHTFPAVLQSSGLYSLSSVVTVPSSSLGTQTYICNVNHKPSNTKVDKKVEPKSCDKTHTSPPSPAPPVAGPSVFLFPPKPKDTLMISRTPEVTCVVVGVSHEDPEVKFNWYVDGVEVHNAKTKPREEQYQSTYRVVSVLTVLHQDWLNGKEYKCKVSNKQLPSPIEKTISKAKGQPSGDIVLTQSPAIMSASPGEKVTMTCSASSSVSYMNWYQQKSGTSPKRWIYDTSKLASGVPAHFRGSGSGTSYSLTISGMEAEDAATYYCQQWSSNPFTFGSGTKLEIN

SEQ ID NO: 101 - protein, 464 aa, Artificial Sequence
  FLT3 x CD3 Fabv
QVQLQQPGAELVKPGASLKLSCKSSGYTFTSYWMHWVRQRPGHGLEWIGEIDPSDSYKDYNQKFKDKATLTVDRSSNTAYMHLSSLTSDDSAVYYCARAITTTPFDFWGQGTTLTVSSASTKGPSVFPLAPSSKSTSGGTAALGCLVKDYFPEPVTVSWNSGALTSGVHTFPAVLQSSGLYSLSSVVTVPSSSLGTQTYICNVNHKPSNTKVDKKVEPKSCDKTHTSPPSPAPPVAGPSVFLFPPKPKDTLMISRTPEVTCVVVGVSHEDPEVKFNWYVDGVEVHNAKTKPREEQYQSTYRVVSVLTVLHQDWLNGKEYKCKVSNKQLPSPIEKTISKAKGQPSGQVQLQQSGAELARPGASVKMSCKASGYTFTRYTMHWVKQRPGQGLEWIGYINPSRGYTNYNQKFKDKATLTTDKSSSTAYMQLSSLTSEDSAVYYCARYYDDHYCLDYWGQGTTLTVSS

SEQ ID NO: 102 - protein, 214 aa, Artificial Sequence
  Anti-FLT3 chimeric light chain (clone 4G8)
DIVLTQSPATLSVTPGDSVSLSCRASQSISNNLHWYQQKSHESPRLLIKYASQSISGIPSRFSGSGSGTDFTLSINSVETEDFGVYFCQQSNTWPYTFGGGTKLEIKRTVAAPSVFIFPPSDEQLKSGTASVVCLLNNFYPREAKVQWKVDNALQSGNSQESVTEQDSKDSTYSLSSTLTLSKADYEKHKVYACEVTHQGLSSPVTKSFNRGEC

SEQ ID NO: 103 - protein, 220 aa, Artificial Sequence
  Anti-FLT3 chimeric light chain (clone BV10)
DIVMTQSPSSLSVSAGEKVTMSCKSSQSLLNSGNQKNYMAWYQQKPGQPPKLLIYGASTRESGVPDRFTGSGSGTDFTLTISSVQAEDLAVYYCQNDHSYPLTFGAGTKLELKRTVAAPSVFIFPPSDEQLKSGTASVVCLLNNFYPREAKVQWKVDNALQSGNSQESVTEQDSKDSTYSLSSTLTLSKADYEKHKVYACEVTHQGLSSPVTKSFNRGEC

SEQ ID NO: 104 - protein, 218 aa, Artificial Sequence
  Anti-CSPG4 chimeric light chain (clone 9.2.27)
DIELTQSPASLAVSLGQRATISCRASESVDSYGNSFMHWYQQKPGQPPKLLIYLASNLESGVPARFSGSGSRTDFTLTIDPVEADDAATYYCQQNNEDPLTFGGGTKLEIKRTVAAPSVFIFPPSDEQLKSGTASVVCLLNNFYPREAKVQWKVDNALQSGNSQESVTEQDSKDSTYSLSSTLTLSKADYEKHKVYACEVTHQGLSSPVTKSFNRGEC

SEQ ID NO: 105 - protein, 219 aa, Artificial Sequence
  Anti-CD19 chimeric light (clone 4G7)
DIVMTQAAPSIPVTPGESVSISCRSSKSLLNSNGNTYLYWFLQRPGQSPQLLIYRMSNLASGVPDRFSGSGSGTAFTLRISRVEAEDVGVYYCMQHLEYPFTFGAGTKLELKRTVAAPSVFIFPPSDEQLKSGTASVVCLLNNFYPREAKVQWKVDNALQSGNSQESVTEQDSKDSTYSLSSTLTLSKADYEKHKVYACEVTHQGLSSPVTKSFNRGEC

SEQ ID NO: 106 - protein, 214 aa, Artificial Sequence
  Anti-EGFR light chain (clone C225)
DILLTQSPVILSVSPGERVSFSCRASQSIGTNIHWYQQRTNGSPRLLIKYASESISGIPSRFSGSGSGTDFTLSINSVESEDIADYYCQQNNNWPTTFGAGTKLELKRTVAAPSVFIFPPSDEQLKSGTASVVCLLNNFYPREAKVQWKVDNALQSGNSQESVTEQDSKDSTYSLSSTLTLSKADYEKHKVYACEVTHQGLSSPVTKSFNRGEC

SEQ ID NO: 107 - DNA, 56 bp, Artificial Sequence
  L1 and further
atgggatggagctggatctttctctttctcctgtcaggaactgcaggtaaggggct

SEQ ID NO: 108 - protein, 15 aa, Artificial Sequence
  L1
MGWSWIFLFLLSGTA

SEQ ID NO: 109 - DNA, 43 bp, Artificial Sequence
  between L1 and L2-VDJ
tgacgtccactctgtctttctcttcacaggtgtcctctcccag

SEQ ID NO: 110 - protein, 4 aa, Artificial Sequence
  L2-VDJ
VLSQ

SEQ ID NO: 111 - DNA, 36 bp, Artificial Sequence
  VDJ ClaI
tcaggtgagtcctaccttctcccattctaaatcgat

SEQ ID NO: 112 - DNA, 35 bp, Artificial Sequence
  MluI-CH1
atcacatacgcgtttttcttgtagcctccaccaag

SEQ ID NO: 113 - DNA, 28 bp, Artificial Sequence
  CH1-BspEI
acccacagggcagccctccggagatatc

SEQ ID NO: 114 - protein, 6 aa, Artificial Sequence
  CH1-BspEI-VL
QPSGDI

SEQ ID NO: 115 - DNA, 20 bp, Artificial Sequence
  VL-SpeI
atcaaatgataactagtccc

SEQ ID NO: 116 - DNA, 35 bp, Artificial Sequence; identical to SEQ ID NO: 112
  MluI-CH1

SEQ ID NO: 117 - DNA, 28 bp, Artificial Sequence
  CH1-BspEI-VH
acccacagggcagccctccggagaggtt

SEQ ID NO: 118 - protein, 6 aa, Artificial Sequence
  CH1-BspEI-VH
QPSGEV

SEQ ID NO: 119 - DNA, 20 bp, Artificial Sequence
  VH-SpeI
tcctcgtgataactagtccc

SEQ ID NO: 120 - DNA, 49 bp, Artificial Sequence
  L1
atggttttcacacctcagatacttggacttatgcttttttggatttcag

SEQ ID NO: 121 - protein, 16 aa, Artificial Sequence
  L1
MVFTPQILGLMLFWIS

SEQ ID NO: 122 - DNA, 12 bp, Artificial Sequence
  between L1 and L2
gtatgactgctt

SEQ ID NO: 123 - DNA, 20 bp, Artificial Sequence
  between L1 and L2
tttccaggtgtccgacgaga

SEQ ID NO: 124 - protein, 4 aa, Artificial Sequence
  L2
ARGD

SEQ ID NO: 125 - DNA, 18 bp, Artificial Sequence
  VJ-SpeI
aaacgtaagtactagttt

SEQ ID NO: 126 - DNA, 41 bp, Artificial Sequence
  Pm1I-CL
cataccatcctcacgtgcttccttcctcagggactgtggct

SEQ ID NO: 127 - DNA, 33 bp, Artificial Sequence
  CL-BsmBI
ggagagtgttagagacaaaggtcctgagacgcc